European Patent Specification EP 3 086 813 B9, published September 27, 2023. Title: SUBSTRATE FOR TRANSGLUTAMINASE. Applicant: COVALAB. The sequence listing filed with the application follows.

SEQUENCE LISTING (33 sequences)

SEQ ID NO: 1 - protein, 6 aa, Artificial Sequence
  Peptide DH6Q5
DVYSQH

SEQ ID NO: 2 - protein, 5 aa, Artificial Sequence
  Peptide FE5Q4
FWIQE

SEQ ID NO: 3 - protein, 6 aa, Artificial Sequence
  Peptide PH6Q4
PLVQSH

SEQ ID NO: 4 - protein, 6 aa, Artificial Sequence
  Peptide PS6Q3
PSVQES

SEQ ID NO: 5 - protein, 7 aa, Artificial Sequence
  Peptide PY7Q5
PLKHQEY

SEQ ID NO: 6 - protein, 12 aa, Artificial Sequence
  Peptide HH12Q11
HDLMWPDVYSQH

SEQ ID NO: 7 - protein, 8 aa, Artificial Sequence
  Peptide WH8Q7
WPDVYSQH

SEQ ID NO: 8 - protein, 8 aa, Artificial Sequence
  Peptide SY10Q8
SPLKHQEY

SEQ ID NO: 9 - protein, 12 aa, Artificial Sequence
  Peptide GS12Q7
GGSPLAQSHGGS

SEQ ID NO: 10 - protein, 12 aa, Artificial Sequence
  Peptide HH12N11
HDLMWPDVYSNH

SEQ ID NO: 11 - protein, 14 aa, Artificial Sequence
  Peptide HG14Q11
HDLMWPDVYSQHGG

SEQ ID NO: 12 - protein, 10 aa, Artificial Sequence
  Peptide WG10Q7
WPDVYSQHGG

SEQ ID NO: 13 - protein, 6 aa, Artificial Sequence
  Peptide DH6N5
DVYSNH

SEQ ID NO: 14 - protein, 13 aa, Artificial Sequence
  Peptide CF13Q4
CYEQHKLPSSWPF

SEQ ID NO: 15 - protein, 9 aa, Artificial Sequence
  Peptide CS9Q4
CYEQHKLPS

SEQ ID NO: 16 - protein, 12 aa, Artificial Sequence
  Peptide FY12Q10
FPWSSPLKHQEY

SEQ ID NO: 17 - protein, 8 aa, Artificial Sequence
  Peptide CW8Q3
CDQMMLPW

SEQ ID NO: 18 - protein, 10 aa, Artificial Sequence
  Peptide YV10
YLADTNSLAV

SEQ ID NO: 19 - protein, 6 aa, Artificial Sequence
  Peptide CV6Q3
CHQSYV

SEQ ID NO: 20 - protein, 6 aa, Artificial Sequence
  Peptide PH6Q4
PLVQSH

SEQ ID NO: 21 - protein, 7 aa, Artificial Sequence
  Peptide VF7Q5
VWRSQYF

SEQ ID NO: 22 - protein, 6 aa, Artificial Sequence
  Peptide DE6Q5
DVYSQE

SEQ ID NO: 23 - protein, 7 aa, Artificial Sequence
  Peptide HL8Q6
HNKSQAL

SEQ ID NO: 24 - protein, 11 aa, Artificial Sequence
  Peptide LN11Q8-10
LLTLPSVQEQN

SEQ ID NO: 25 - protein, 11 aa, Artificial Sequence
  Peptide LN11Q10
LLTLPSVSEQN

SEQ ID NO: 26 - protein, 7 aa, Artificial Sequence
  Peptide KL7Q5
KEEFQPL

SEQ ID NO: 27 - protein, 8 aa, Artificial Sequence
  Peptide SY8Q6
SPLKHQEY

SEQ ID NO: 28 - protein, 7 aa, Artificial Sequence
  Peptide WD7Q7
WPLMMQD

SEQ ID NO: 29 - protein, 5 aa, Artificial Sequence
  synthetic peptide
YEIQR

SEQ ID NO: 30 - protein, 5 aa, Artificial Sequence
  synthetic peptide
YEAQK

SEQ ID NO: 31 - protein, 5 aa, Artificial Sequence
  synthetic peptide
YEAQR

SEQ ID NO: 32 - protein, 5 aa, Artificial Sequence
  synthetic peptide
WPAQR

SEQ ID NO: 33 - protein, 5 aa, Artificial Sequence
  synthetic peptide
YEVQK